European Patent Specification EP 3 755 814 B1, published April 9, 2025. Title: ASSAY FOR DETECTION OF ANDROGEN RECEPTOR VARIANTS. Applicant: Giannakakou, Paraskevi Ph.D. Gjyrezi, Ada Kim, Seaho. The sequence listing filed with the application follows.

SEQUENCE LISTING (17 sequences)

SEQ ID NO: 1 - protein, 919 aa, Homo sapiens
MEVQLGLGRVYPRPPSKTYRGAFQNLFQSVREVIQNPGPRHPEAASAAPPGASLLLLQQQQQQQQQQQQQQQQQQQQQETSPRQQQQQQGEDGSPQAHRRGPTGYLVLDEEQQPSQPQSALECHPERGCVPEPGAAVAASKGLPQQLPAPPDEDDSAAPSTLSLLGPTFPGLSSCSADLKDILSEASTMQLLQQQQQEAVSEGSSSGRAREASGAPTSSKDNYLGGTSTISDNAKELCKAVSVSMGLGVEALEHLSPGEQLRGDCMYAPLLGVPPAVRPTPCAPLAECKGSLLDDSAGKSTEDTAEYSPFKGGYTKGLEGESLGCSGSAAAGSSGTLELPSTLSLYKSGALDEAAAYQSRDYYNFPLALAGPPPPPPPPHPHARIKLENPLDYGSAWAAAAAQCRYGDLASLHGAGAAGPGSGSPSAAASSSWHTLFTAEEGQLYGPCGGGGGGGGGGGGGGGGGGGGGGGGEAGAVAPYGYTRPPQGLAGQESDFTAPDVWYPGGMVSRVPYPSPTCVKSEMGPWMDSYSGPYGDMRLETARDHVLPIDYYFPPQKTCLICGDEASGCHYGALTCGSCKVFFKRAAEGKQKYLCASRNDCTIDKFRRKNCPSCRLRKCYEAGMTLGARKLKKLGNLKLQEEGEASSTTSPTEETTQKLTVSHIEGYECQPIFLNVLEAIEPGVVCAGHDNNQPDSFAALLSSLNELGERQLVHVVKWAKALPGFRNLHVDDQMAVIQYSWMGLMVFAMGWRSFTNVNSRMLYFAPDLVFNEYRMHKSRMYSQCVRMRHLSQEFGWLQITPQEFLCMKALLLFSIIPVDGLKNQKFFDELRMNYIKELDRIIACKRKNPTSCSRRFYQLTKLLDSVQPIARELHQFTFDLLIKSHMVSVDFPEMMAEIISVQVPKILSGKVKPIYFHTQ

SEQ ID NO: 2 - DNA, 3568 bp, Homo sapiens
taataactcagttcttatttgcacctacttcagtggacactgaatttggaaggtggaggattttgtttttttcttttaagatctgggcatcttttgaatctacccttcaagtattaagagacagactgtgagcctagcagggcagatcttgtccaccgtgtgtcttcttctgcacgagactttgaggctgtcagagcgctttttgcgtggttgctcccgcaagtttccttctctggagcttcccgcaggtgggcagctagctgcagcgactaccgcatcatcacagcctgttgaactcttctgagcaagagaaggggaggcggggtaagggaagtaggtggaagattcagccaagctcaaggatggaagtgcagttagggctgggaagggtctaccctcggccgccgtccaagacctaccgaggagctttccagaatctgttccagagcgtgcgcgaagtgatccagaacccgggccccaggcacccagaggccgcgagcgcagcacctcccggcgccagtttgctgctgctgcagcagcagcagcagcagcagcagcagcagcagcagcagcagcagcagcagcagcagcagcaagagactagccccaggcagcagcagcagcagcagggtgaggatggttctccccaagcccatcgtagaggccccacaggctacctggtcctggatgaggaacagcaaccttcacagccgcagtcggccctggagtgccaccccgagagaggttgcgtcccagagcctggagccgccgtggccgccagcaaggggctgccgcagcagctgccagcacctccggacgaggatgactcagctgccccatccacgttgtccctgctgggccccactttccccggcttaagcagctgctccgctgaccttaaagacatcctgagcgaggccagcaccatgcaactccttcagcaacagcagcaggaagcagtatccgaaggcagcagcagcgggagagcgagggaggcctcgggggctcccacttcctccaaggacaattacttagggggcacttcgaccatttctgacaacgccaaggagttgtgtaaggcagtgtcggtgtccatgggcctgggtgtggaggcgttggagcatctgagtccaggggaacagcttcggggggattgcatgtacgccccacttttgggagttccacccgctgtgcgtcccactccttgtgccccattggccgaatgcaaaggttctctgctagacgacagcgcaggcaagagcactgaagatactgctgagtattcccctttcaagggaggttacaccaaagggctagaaggcgagagcctaggctgctctggcagcgctgcagcagggagctccgggacacttgaactgccgtctaccctgtctctctacaagtccggagcactggacgaggcagctgcgtaccagagtcgcgactactacaactttccactggctctggccggaccgccgccccctccgccgcctccccatccccacgctcgcatcaagctggagaacccgctggactacggcagcgcctgggcggctgcggcggcgcagtgccgctatggggacctggcgagcctgcatggcgcgggtgcagcgggacccggttctgggtcaccctcagccgccgcttcctcatcctggcacactctcttcacagccgaagaaggccagttgtatggaccgtgtggtggtggtgggggtggtggcggcggcggcggcggcggcggcggcggcggcggcggcggcggcggcggcggcgaggcgggagctgtagccccctacggctacactcggccccctcaggggctggcgggccaggaaagcgacttcaccgcacctgatgtgtggtaccctggcggcatggtgagcagagtgccctatcccagtcccacttgtgtcaaaagcgaaatgggcccctggatggatagctactccggaccttacggggacatgcgtttggagactgccagggaccatgttttgcccattgactattactttccaccccagaagacctgcctgatctgtggagatgaagcttctgggtgtcactatggagctctcacatgtggaagctgcaaggtcttcttcaaaagagccgctgaagggaaacagaagtacctgtgcgccagcagaaatgattgcactattgataaattccgaaggaaaaattgtccatcttgtcgtcttcggaaatgttatgaagcagggatgactctgggagcccggaagctgaagaaacttggtaatctgaaactacaggaggaaggagaggcttccagcaccaccagccccactgaggagacaacccagaagctgacagtgtcacacattgaaggctatgaatgtcagcccatctttctgaatgtcctggaagccattgagccaggtgtagtgtgtgctggacacgacaacaaccagcccgactcctttgcagccttgctctctagcctcaatgaactgggagagagacagcttgtacacgtggtcaagtgggccaaggccttgcctggcttccgcaacttacacgtggacgaccagatggctgtcattcagtactcctggatggggctcatggtgtttgccatgggctggcgatccttcaccaatgtcaactccaggatgctctacttcgcccctgatctggttttcaatgagtaccgcatgcacaagtcccggatgtacagccagtgtgtccgaatgaggcacctctctcaagagtttggatggctccaaatcaccccccaggaattcctgtgcatgaaagcactgctactcttcagcattattccagtggatgggctgaaaaatcaaaaattctttgatgaacttcgaatgaactacatcaaggaactcgatcgtatcattgcatgcaaaagaaaaaatcccacatcctgctcaagacgcttctaccagctcaccaagctcctggactccgtgcagcctattgcgagagagctgcatcagttcacttttgacctgctaatcaagtcacacatggtgagcgtggactttccggaaatgatggcagagatcatctctgtgcaagtgcccaagatcctttctgggaaagtcaagcccatctatttccacacccagtgaagcattggaaaccctatttccccaccccagctcatgccccctttcagatgtcttctgcctgttataactctgcactactcctctgcagtgccttggggaatttcctctattgatgtacagtctgtcatgaacatgttcctgaattctatttgctgggctttttttttctctttctctcctttctttttcttcttccctccctatctaaccctcccatggcaccttcagactttgcttcccattgtggctcctatctgtgttttgaatggtgttgtatgctttaaatctgtgatgatcctcatatggcccagtgtcaagttgtgcttgtttacagcactactctgtgccagccacacaaacgtttacttatcttatgccacgggaagtttagagagctaagattatctggggaaatcaaaacaaaaaacaagcaaacaaaaaaaaaa

SEQ ID NO: 3 - protein, 739 aa, Homo sapiens
MEVQLGLGRVYPRPPSKTYRGAFQNLFQSVREVIQNPGPRHPEAASAAPPGASLLLLQQQQQQQQQQQQQQQQQQQQQQQQETSPRQQQQQQGEDGSPQAHRRGPTGYLVLDEEQQPSQPQSALECHPERGCVPEPGAAVAASKGLPQQLPAPPDEDDSAAPSTLSLLGPTFPGLSSCSADLKDILSEASTMQLLQQQQQEAVSEGSSSGRAREASGAPTSSKDNYLGGTSTISDNAKELCKAVSVSMGLGVEALEHLSPGEQLRGDCMYAPLLGVPPAVRPTPCAPLAECKGSLLDDSAGKSTEDTAEYSPFKGGYTKGLEGESLGCSGSAAAGSSGTLELPSTLSLYKSGALDEAAAYQSRDYYNFPLALAGPPPPPPPPHPHARIKLENPLDYGSAWAAAAAQCRYGDLASLHGAGAAGPGSGSPSAAASSSWHTLFTAEEGQLYGPCGGGGGGGGGGGGGGGGGGGGGGGGGGGEAGAVAPYGYTRPPQGLAGQESDFTAPDVWYPGGMVSRVPYPSPTCVKSEMGPWMDSYSGPYGDMRLETARDHVLPIDYYFPPQKTCLICGDEASGCHYGALTCGSCKVFFKRAAEGKQKYLCASRNDCTIDKFRRKNCPSCRLRKCYEAGMTLGARKLKKLGNLKLQEEGEASSTTSPTEETTQKLTVSHIEGYECQPIFLNVLEAIEPGVVCAGHDNNQPDSFAALLSSLNELGERQLVHVVKWAKALPDCERAASVHF

SEQ ID NO: 4 - DNA, 2442 bp, Homo sapiens
aggatggaagtgcagttagggctgggaagggtctaccctcggccgccgtccaagacctaccgaggagctttccagaatctgttccagagcgtgcgcgaagtgatccagaacccgggccccaggcacccagaggccgcgagcgcagcacctcccggcgccagtttgctgctgctgcagcagcagcagcagcagcagcagcagcagcagcagcagcagcagcagcagcagcagcagcagcagcagcaagagactagccccaggcagcagcagcagcagcagggtgaggatggttctccccaagcccatcgtagaggccccacaggctacctggtcctggatgaggaacagcaaccttcacagccgcagtcggccctggagtgccaccccgagagaggttgcgtcccagagcctggagccgccgtggccgccagcaaggggctgccgcagcagctgccagcacctccggacgaggatgactcagctgccccatccacgttgtccctgctgggccccactttccccggcttaagcagctgctccgctgaccttaaagacatcctgagcgaggccagcaccatgcaactccttcagcaacagcagcaggaagcagtatccgaaggcagcagcagcgggagagcgagggaggcctcgggggctcccacttcctccaaggacaattacttagggggcacttcgaccatttctgacaacgccaaggagttgtgtaaggcagtgtcggtgtccatgggcctgggtgtggaggcgttggagcatctgagtccaggggaacagcttcggggggattgcatgtacgccccacttttgggagttccacccgctgtgcgtcccactccttgtgccccattggccgaatgcaaaggttctctgctagacgacagcgcaggcaagagcactgaagatactgctgagtattcccctttcaagggaggttacaccaaagggctagaaggcgagagcctaggctgctctggcagcgctgcagcagggagctccgggacacttgaactgccgtctaccctgtctctctacaagtccggagcactggacgaggcagctgcgtaccagagtcgcgactactacaactttccactggctctggccggaccgccgccccctccgccgcctccccatccccacgctcgcatcaagctggagaacccgctggactacggcagcgcctgggcggctgcggcggcgcagtgccgctatggggacctggcgagcctgcatggcgcgggtgcagcgggacccggttctgggtcaccctcagccgccgcttcctcatcctggcacactctcttcacagccgaagaaggccagttgtatggaccgtgtggtggtggtgggggtggtggcggcggcggcggcggcggcggcggcggcggcggcggcggcggcggcggcggcggcggcggcgaggcgggagctgtagccccctacggctacactcggccccctcaggggctggcgggccaggaaagcgacttcaccgcacctgatgtgtggtaccctggcggcatggtgagcagagtgccctatcccagtcccacttgtgtcaaaagcgaaatgggcccctggatggatagctactccggaccttacggggacatgcgtttggagactgccagggaccatgttttgcccattgactattactttccaccccagaagacctgcctgatctgtggagatgaagcttctgggtgtcactatggagctctcacatgtggaagctgcaaggtcttcttcaaaagagccgctgaagggaaacagaagtacctgtgcgccagcagaaatgattgcactattgataaattccgaaggaaaaattgtccatcttgtcgtcttcggaaatgttatgaagcagggatgactctgggagcccggaagctgaagaaacttggtaatctgaaactacaggaggaaggagaggcttccagcaccaccagccccactgaggagacaacccagaagctgacagtgtcacacattgaaggctatgaatgtcagcccatctttctgaatgtcctggaagccattgagccaggtgtagtgtgtgctggacacgacaacaaccagcccgactcctttgcagccttgctctctagcctcaatgaactgggagagagacagcttgtacacgtggtcaagtgggccaaggccttgcctgattgcgagagagctgcatcagttcacttttgacctgctaatcaagtcacacatggtgagcgtggactttccggaaatgatggcagagatcatctctgtgcaagtgcccaagatcctttctgggaaagtcaagcccatctatttccacacccagtgaagcattggaaaccctatttccccaccccagctcatgccccctttcagatgtcttctgcctgttataactctgcactactcctctgcagtgccttg

SEQ ID NO: 5 - protein, 645 aa, Homo sapiens
MEVQLGLGRVYPRPPSKTYRGAFQNLFQSVREVIQNPGPRHPEAASAAPPGASLLLQQQQQQQQQQQQQQQQQQQQQQQQQQQQQETSPRQQQQQQGEDGSPQAHRRGPTGYLVLDEEQQPSQPQSALECHPERGCVPEPGAAVAASKGLPQQLPAPPDEDDSAAPSTLSLLGPTFPGLSSCSADLKDILSEASTMQLLQQQQQEAVSEGSSSGRAREASGAPTSSKDNYLGGTSTISDNAKELCKAVSVSMGLGVEALEHLSPGEQLRGDCMYAPLLGVPPAVRPTPCAPLAECKGSLLDDSAGKSTEDTAEYSPFKGGYTKGLEGESLGCSGSAAAGSSGTLELPSTLSLYKSGALDEAAAYQSRDYYNFPLALAGPPPPPPPPHPHARIKLENPLDYGSAWAAAAAQCRYGDLASLHGAGAAGPGSGSPSAAASSSWHTLFTAEEGQLYGPCGGGGGGGGGGGGGGGGGGGEAGAVAPYGYTRPPQGLAGQESDFTAPDVWYPGGMVSRVPYPSPTCVKSEMGPWMDSYSGPYGDMRLETARDHVLPIDYYFPPQKTCLICGDEASGCHYGALTCGSCKVFFKRAAEGKQKYLCASRNDCTIDKFRRKNCPSCRLRKCYEAGMTLGEKFRVGNCKHLKMTRP

SEQ ID NO: 6 - DNA, 3641 bp, Homo sapiens
gacactgaatttggaaggtggaggattttgtttttttcttttaagatctgggcatcttttgaatctacccttcaagtattaagagacagactgtgagcctagcagggcagatcttgtccaccgtgtgtcttcttctgcacgagactttgaggctgtcagagcgctttttgcgtggttgctcccgcaagtttccttctctggagcttcccgcaggtgggcagctagctgcagcgactaccgcatcatcacagcctgttgaactcttctgagcaagagaaggggaggcggggtaagggaagtaggtggaagattcagccaagctcaaggatggaagtgcagttagggctgggaagggtctaccctcggccgccgtccaagacctaccgaggagctttccagaatctgttccagagcgtgcgcgaagtgatccagaacccgggccccaggcacccagaggccgcgagcgcagcacctcccggcgccagtttgctgctgcagcagcagcagcagcagcagcagcagcagcagcagcagcagcagcagcagcagcagcagcagcagcagcagcagcagcagcagcaagagactagccccaggcagcagcagcagcagcagggtgaggatggttctccccaagcccatcgtagaggccccacaggctacctggtcctggatgaggaacagcaaccttcacagccgcagtcggccctggagtgccaccccgagagaggttgcgtcccagagcctggagccgccgtggccgccagcaaggggctgccgcagcagctgccagcacctccggacgaggatgactcagctgccccatccacgttgtccctgctgggccccactttccccggcttaagcagctgctccgctgaccttaaagacatcctgagcgaggccagcaccatgcaactccttcagcaacagcagcaggaagcagtatccgaaggcagcagcagcgggagagcgagggaggcctcgggggctcccacttcctccaaggacaattacttagggggcacttcgaccatttctgacaacgccaaggagttgtgtaaggcagtgtcggtgtccatgggcctgggtgtggaggcgttggagcatctgagtccaggggaacagcttcggggggattgcatgtacgccccacttttgggagttccacccgctgtgcgtcccactccttgtgccccattggccgaatgcaaaggttctctgctagacgacagcgcaggcaagagcactgaagatactgctgagtattcccctttcaagggaggttacaccaaagggctagaaggcgagagcctaggctgctctggcagcgctgcagcagggagctccgggacacttgaactgccgtctaccctgtctctctacaagtccggagcactggacgaggcagctgcgtaccagagtcgcgactactacaactttccactggctctggccggaccgccgccccctccgccgcctccccatccccacgctcgcatcaagctggagaacccgctggactacggcagcgcctgggcggctgcggcggcgcagtgccgctatggggacctggcgagcctgcatggcgcgggtgcagcgggacccggttctgggtcaccctcagccgccgcttcctcatcctggcacactctcttcacagccgaagaaggccagttgtatggaccgtgtggtggtggtgggggtggtggcggcggcggcggcggcggcggcggcggcggcggcggcgaggcgggagctgtagccccctacggctacactcggccccctcaggggctggcgggccaggaaagcgacttcaccgcacctgatgtgtggtaccctggcggcatggtgagcagagtgccctatcccagtcccacttgtgtcaaaagcgaaatgggcccctggatggatagctactccggaccttacggggacatgcgtttggagactgccagggaccatgttttgcccattgactattactttccaccccagaagacctgcctgatctgtggagatgaagcttctgggtgtcactatggagctctcacatgtggaagctgcaaggtcttcttcaaaagagccgctgaagggaaacagaagtacctgtgcgccagcagaaatgattgcactattgataaattccgaaggaaaaattgtccatcttgtcgtcttcggaaatgttatgaagcagggatgactctgggagaaaaattccgggttggcaattgcaagcatctcaaaatgaccagaccctgaagaaaggctgacttgcctcattcaaaatgagggctctagagggctctagtggatagtctggagaaacctggcgtctgaggcttaggagcttaggtttttgctcctcaacacagactttgacgttggggttgggggctactctcttgattgctgactccctccagcgggaccaatagtgttttcctacctcacagggatgttgtgaggacgggctgtagaagtaatagtggttaccactcatgtagttgtgagtatcatgattattgtttcctgtaatgtggcttggcattggcaaagtgctttttgattgttcttgatcacatatgatgggggccaggcactgactcaggcggatgcagtgaagctctggctcagtcgcttgcttttcgtggtgtgctgccaggaagaaactttgctgatgggactcaaggtgtcaccttggacaagaagcaactgtgtctgtctgaggttcctgtggccatctttatttgtgtattaggcaattcgtatttcccccttaggttctagccttctggatcccagccagtgacctagatcttagcctcaggccctgtcactgagctgaaggtagtagctgatccacagaagttcagtaaacaaggaccagatttctgcttctccaggagaagaagccagccaacccctctcttcaaacacactgagagactacagtccgactttccctcttacatctagccttactgtagccacactccttgattgctctctcacatcacatgcttctcttcatcagttgtaagcctctcattcttctcccaagccagactcaaatattgtattgatgtcaaagaagaatcacttagagtttggaatatcttgttctctctctgctccatagcttccatattgacaccagtttctttctagtggagaagtggagtctgtgaagccagggaaacacacatgtgagagtcagaaggactctccctgacttgcctggggcctgtctttcccaccttctccagtctgtctaaacacacacacacacacacacacacacacacacacacacacacacgctctctctctctctccccccccaacacacacacactctctctctcacacacacacacatacacacacacttctttctctttcccctgactcagcaacattctggagaaaagccaaggaaggacttcaggaggggagtttcccccttctcagggcagaattttaatctccagaccaacaagaagttccctaatgtggattgaaaggctaatgaggtttatttttaactactttctatttgtttgaatgttgcatatttctactagtgaaattttcccttaataaagccattaatacacccaaaaaaaaaaaaaaaa

SEQ ID NO: 7 - DNA, 20 bp, Artificial Sequence
  A synthetic oligonucleotide
aatcccacatcctgctcaag

SEQ ID NO: 8 - DNA, 19 bp, Artificial Sequence
  A synthetic oligonucleotide
gcagcctattgcgagagag

SEQ ID NO: 9 - DNA, 21 bp, Artificial Sequence
  A synthetic oligonucleotide
accagctcaccaagctcctgg

SEQ ID NO: 10 - skipped

SEQ ID NO: 11 - DNA, 20 bp, Artificial Sequence
  A synthetic oligonucleotide
agggatgactctgggagaaa

SEQ ID NO: 12 - DNA, 20 bp, Artificial Sequence
  A synthetic oligonucleotide
aaaggctgacttgcctcatt

SEQ ID NO: 13 - DNA, 21 bp, Artificial Sequence
  A synthetic oligonucleotide
tccgggttggcaattgcaagc

SEQ ID NO: 14 - skipped

SEQ ID NO: 15 - DNA, 20 bp, Artificial Sequence
  A synthetic oligonucleotide
ctttgcagccttgctctcta

SEQ ID NO: 16 - DNA, 20 bp, Artificial Sequence
  A synthetic oligonucleotide
cttgcctgattgcgagagag

SEQ ID NO: 17 - DNA, 20 bp, Artificial Sequence
  A synthetic oligonucleotide
acacgtggtcaagtgggcca